European Patent Specification EP 4 004 056 B1, published September 24, 2025. Title: BINDING MEMBERS. Applicant: Scancell Limited. The sequence listing filed with the application follows.

SEQUENCE LISTING (22 sequences)

SEQ ID NO: 1 - DNA, 1401 bp, Artificial sequence
  Heavy chain DNA sequence of 27.10
atgaacttctggctcagcttgattttccttgtccttgttttaaaaggtgtccagtgtgaagtgaagctggtggagtctgggggaggcttagtgcagcctggagggtccctgaaactctcctgtgcaacctctggattcactttcagtcactattacatgtattgggttcgccagactccagagaagaggctggagtgggtcgcatacattagtaatgatggtgataacacctattatccagacactataaggggccgattcaccatctccagagacaatgccaggaacaccctgtacctgcaaatgagccgtctgaagtctgaggacacagccatgtattactgtgcaagagggaagtacgacggggcctggtttgcttactggggccaagggactctggtcactgtctctgcagctacaacaacagccccatctgtctatcccttggtccctggctgcagtgacacatctggatcctcggtgacactgggatgccttgtcaaaggctacttccctgagccggtaactgtaaaatggaactatggagccctgtccagcggtgtgcgcacagtctcatctgtcctgcagtctgggttctattccctcagcagcttggtgactgtaccctccagcacctggcccagccagactgtcatctgcaacgtagcccacccagccagcaagactgagttgatcaagagaatcgagcctagaatacccaagcccagtacccccccaggttcttcatgcccacctggtaacatcttgggtggaccatccgtcttcatcttccccccaaagcccaaggatgcactcatgatctccctaacccccaaggttacgtgtgtggtggtggatgtgagcgaggatgacccagatgtccatgtcagctggtttgtggacaacaaagaagtacacacagcctggacacagccccgtgaagctcagtacaacagtaccttccgagtggtcagtgccctccccatccagcaccaggactggatgaggggcaaggagttcaaatgcaaggtcaacaacaaagccctcccagcccccatcgagagaaccatctcaaaacccaaaggaagagcccagacacctcaagtatacaccatacccccacctcgtgaacaaatgtccaagaagaaggttagtctgacctgcctggtcaccaacttcttctctgaagccatcagtgtggagtgggaaaggaacggagaactggagcaggattacaagaacactccacccatcctggactcagatgggacctacttcctctacagcaagctcactgtggatacagacagttggttgcaaggagaaatttttacctgctccgtggtgcatgaggctctccataaccaccacacacagaagctgtctcgctcccctggtaaa

SEQ ID NO: 2 - protein, 465 aa, Artificial sequence
  Heavy chain protein sequence of 27.10
MNFWLSLIFLVLVLKGVQCEVKLVESGGGLVQPGGSLKLSCATSGFTFYYMYWVRQTPEKRLEWVAYISNDDNTYYPDTIRGRFTISRDNARNTLYLQMSRLKSEDTAMYYCARGKYDGAWFAYWGQGTLVTVSAATTTAPSVYPLVPGCSDTSGSSVTLGCLVKGYFPEPVTVKWNYGALSSGVRTVSSVLQSGFYSLSSLVTVPSSTWPSQTVICNVAHPASKTELIKRIEPRIPKPSTPPGSSCPPGNILGGPSVFIFPPKPKDALMISLTPKVTCVVVDVSEDDPDVHVSWFVDNKEVHTAWTQPREAQYNSTFRVVSALPIQHQDWMRGKEFKCKVNNKALPAPIERTISKPKGRAQTPQVYTIPPPREQMSKKKVSLTCLVTNFFSEAISVEWERNGELEQDYKNTPPILDSDGTYFLYSKLTVDTDSWLQGEIFTCSVVHEALHNHHTQKNLSRSPGK

SEQ ID NO: 3 - DNA, 1386 bp, Artificial sequence
  Heavy chain DNA sequence of 27.18
atgaacttctggctcagcttgattttccttgtccttgttttaaaaggtgtccagtgtgaagtgaagctggtggagtctgggggaggcttagtgcagcctggagggtccctgaaactctcctgtgcaacctctggattcactttcagtcactattacatgtattgggttcgccagactccagagaagaggctggagtgggtcgcatacattagtaatgatggtgataacacctattatccagacactataaggggccgattcaccatctccagagacaatgccaggaacaccctgtacctgcaaatgagccgtctgaagtctgaggacacagccatgtattactgtgcaagagggaagtacgacggggcctggtttgcttactggggccaagggactctggtcactgtctctgcagccaaaacgacacccccatctgtctatccactggcccctggatctgctgcccaaactaactccatggtgaccctgggatgcctggtcaagggctatttccctgagccagtgacagtgacctggaactctggatccctgtccagcggtgtgcacaccttcccagctgtcctggagtctgacctctacactctgagcagctcagtgactgtcccctccagccctcggcccagcgagaccgtcacctgcaacgttgcccacccggccagcagcaccaaggtggacaagaaaattgtgcccagggattgtggttgtaagccttgcatatgtacagtcccagaagtatcatctgtcttcatcttccccccaaagcccaaggatgtgctcaccattactctgactcctaaggtcacgtgtgttgtggtagacatcagcaaggatgatcccgaggtccagttcagctggtttgtagatgatgtggaggtgcacacagctcagacgcaaccccgggaggagcagttcaacagcactttccgctcagtcagtgaacttcccatcatgcaccaggactggctcaatggcaaggagttcaaatgcagggtcaacagtgcagctttccctgcccccatcgagaaaaccatctccaaaaccaaaggcagaccgaaggctccacaggtgtacaccattccacctcccaaggagcagatggccaaggataaagtcagtctgacctgcatgataacagacttcttccctgaagacattactgtggagtggcagtggaatgggcagccagcggagaactacaagaacactcagcccatcatgaacacgaatggctcttacttcgtctacagcaagctcaatgtgcagaagagcaactgggaggcaggaaatactttcacctgctctgtgttacatgagggcctgcacaaccaccatactgagaagagcctctcccactctcctggtaaa

SEQ ID NO: 4 - protein, 461 aa, Artificial sequence
  Heavy chain protein sequence of 27.18
MNFWLSLIFLVLVLKGVQCEVKLVESGGGLVQPGGSLKLSCATSGFTFHYYMYWVRQTPEKRLEWVAYISNDGDNTYYPDTIRGRFTISRDNARNTLYLQMSRLKSEDTAMYYCARGKYDGAWFAYWGQGTLVTVSAAKTTPPSVYPLAPGSAAQTNSMVTLGCLVKGYFPEPVTVTWNSGSLSSGVHTFPAVLESDLYTLSSSVTVPSSPRPSETVTCNVAHPASSTKVDKKIVPRDCGCKPCICTVPEVSSVFIFPPKPKDVLTITLTPKVTCVVVDISKDDPEVQFSWFVDDVEVHTAQTQPREEQFNSTFRSVSELPIMHQDWLNGKEFKCRVNSAAFPAPIEKTISKTKGRPKAPQVYTIPPPKEQMAKDKVSLTCMITDFFPEDITVEWQWNGQPAENYKNTQPIMNTNGSYFVYSKLNVQKSNWEAGNTFTCSVLHEGLHNHHTEKSLSHSPGK

SEQ ID NO: 5 - DNA, 714 bp, Artificial sequence
  Light chain DNA sequence FG27.10
atgaagttgcctgttaggctgttggtgctgatgttctggattcctgcttccatcagtgatgttttgatgacccaaactccactctccctgcctgtcagtcttggagatcaagcctccatctcttgcagatctagtcagatcattgtacatactaatggaaacacctatttagaatggtacctgcagaaaccaggccagtctccaaacctcctgatctacaaagtttccaaccgattttctggggtcccagacaggttcagtggcagtggatcagggacagatttcacactcaagatcagcagagtggaggctgaggatctgggagtttattactgctttcaaggttcacatgttccattcacgttcggctcggggacaaagttggaaataaaacgggctgatgctgcaccaactgtatccatcttcccaccatccagtgagcagttaacatctggaggtgcctcagtcgtgtgcttcttgaacaacttctaccccaaagacatcaatgtcaagtggaagattgatggcagtgaacgacaaaatggcgtcctgaacagttggactgatcaggacagcaaagacagcacctacagcatgagcagcaccctcacgttgaccaaggacgagtatgaacgacataacagctatacctgtgaggccactcacaagacatcaacttcacccattgtcaagagcttcaacaggaatgagtgt

SEQ ID NO: 6 - protein, 238 aa, Artificial sequence
  Light chain protein sequence FG27.10
MKLPVRLLVLMFWIPASISDVLMTQTPLSLPVSLGDQASISCRSSQIIVHTNGNTYLEWYLQKPGQSPNLLIYKVSNRFSGVPDRFSGSGSGTDFTLKISRVEAEDLGVYYCFQGSHVPFTFGSGTKLEIKRADAAPTVSIFPPSSEQLTSGGASVVCFLNNFYPKDINVKWKIDGSERQNGVLNSWTDQDSKDSTYSMSSTLTLTKDEYERHNSYTCEATHKTSTSPIVKSFNRNEC

SEQ ID NO: 7 - DNA, 1404 bp, Artificial sequence
  Heavy chain DNA sequence CH27.10
atgaacttctggctcagcttgattttccttgtccttgttttaaaaggtgtccagtgtgaagtgaagctggtggagtctgggggaggcttagtgcagcctggagggtccctgaaactctcctgtgcaacctctggattcactttcagtcactattacatgtattgggttcgccagactccagagaagaggctggagtgggtcgcatacattagtaatgatggtgataacacctattatccagacactataaggggccgattcaccatctccagagacaatgccaggaacaccctgtacctgcaaatgagccgtctgaagtctgaggacacagccatgtattactgtgcaagagggaagtacgacggggcctggtttgcttactggggccaagggactctggtcactgtctctagcgcttccaccaagggcccatcggtcttccccctggcaccctcctccaagagcacctctgggggcacagcggccctgggctgcctggtcaaggactacttccccgaaccggtgacggtgtcgtggaactcaggcgccctgaccagcggcgtgcacaccttcccggctgtcctacagtcctcaggactctactccctcagcagcgtggtgaccgtgccctccagcagcttgggcacccagacctacatctgcaacgtgaatcacaagcccagcaacaccaaggtggacaagaaagttgagcccaaatcttgtgacaaaactcacacatgcccaccgtgcccagcacctgaactcctggggggaccgtcagtcttcctcttccccccaaaacccaaggacaccctcatgatctcccggacccctgaggtcacatgcgtggtggtggacgtgagccacgaagaccctgaggtcaagttcaactggtacgtggacggcgtggaggtgcataatgccaagacaaagccgcgggaggagcagtacaacagcacgtaccgtgtggtcagcgtcctcaccgtcctgcaccaggactggctgaatggcaaggagtacaagtgcaaggtctccaacaaagccctcccagcccccatcgagaaaaccatctccaaagccaaagggcagccccgagaaccacaggtgtacaccctgcccccatcccgggatgagctgaccaagaaccaggtcagcctgacctgcctggtcaaaggcttctatcccagcgacatcgccgtggagtgggagagcaatgggcagccggagaacaactacaagaccacgcctcccgtgctggactccgacggctccttcttcctctacagcaagctcaccgtggacaagagcaggtggcagcaggggaacgtcttctcatgctccgtgatgcatgaggctctgcacaaccactacacgcagaagagcctctccctgtctccgggtaaa

SEQ ID NO: 8 - protein, 467 aa, Artificial sequence
  Heavy chain protein sequence CH27.10
MNFWLSLIFLVLVLKGVQCEVKLVESGGGLVQPGGSLKLSCATSGFTFHYYMYWVRQTPEKRLEWVAYISNDGDNTYYPDTIRGRFTISRDNARNTLYLQMSRLKSEDTAMYYCARGKYDGAWFAYWGQGTLVTVSSASTKGPSVFPLAPSSKSTSGGTAALGCLVKDYFPEPVTVSWNSGALTSGVHTFPAVLQSSGLYSLSSVVTVPSSSLGTQTYICNVNHKPSNTKVDKKVEPKSCDKTHTCPPCPAPELLGGPSVFLFPPKPKDTLMISRTPEVTCVVVDVSHEDPEVKFNWYVDGVEVHNAKTKPREEQYNSTYRVVSVLTVLHQDWLNGKEYKCKVSNKALPAPIEKTISKAKGQPREPQVYTLPPSRDELTKNQVSLTCLVKGFYPSDIAVEWESNGQPENNYKTTPPVLDSDGSFFLYSKLTVDKSRWQQGNVFSCSVMHEALHNHYTQKSLSLSPGK

SEQ ID NO: 9 - DNA, 714 bp, Artificial sequence
  CH27.10 light chain DNA sequence
atgaagttgcctgttaggctgttggtgctgatgttctggattcctgcttccatcagtgatgttttgatgacccaaactccactctccctgcctgtcagtcttggagatcaagcctccatctcttgcagatctagtcagatcattgtacatactaatggaaacacctatttagaatggtacctgcagaaaccaggccagtctccaaacctcctgatctacaaagtttccaaccgattttctggggtcccagacaggttcagtggcagtggatcagggacagatttcacactcaagatcagcagagtggaggctgaggatctgggagtttattactgctttcaaggttcacatgttccattcacgttcggctcggggacaaagttggaaataaaacgtacggtagcggccccatctgtcttcatcttcccgccatctgatgagcagttgaaatctggaactgcctctgttgtgtgcctgctgaataacttctatcccagagaggccaaagtacagtggaaggtggataacgccctccaatcgggtaactcccaggagagtgtcacagagcaggacagcaaggacagcacctacagcctcagcagcaccctgacgctgagcaaagcagactacgagaaacacaaagtctacgcctgcgaagtcacccatcagggcctgagctcgcccgtcacaaagagcttcaacaggggagagtgt

SEQ ID NO: 10 - protein, 238 aa, Artificial sequence
  CH27.10 light chain protein sequence
MKLPVRLLVLMFWIPASISDVLMTQTPLSLPVSLGDQASISCRSSQIIVHTNGNTYLEWYLQKPGQSPNLLIYKVSNRFSGVPDRFSGSGSGTDFTLKISRVEAEDLGVYYCFQGSHVPFTFGSGTKLEIKRTVAAPSVFIFPPSDEQLKSGTASVVCLLNNFYPREAKVQWKVDNALQSGNSQESVTEQDSKDSTYSLSSTLTLSKADYEKHKVYACEVTHQGLSSPVTKSFNRGEC

SEQ ID NO: 11 - DNA, 357 bp, Artificial sequence
  FG27 RHA
caggtccagctggtcgaatcagggggaggcgtcgtgcagcccggaaggtcactgagactgtcatgtgccgcatcagggtttactttctcacactactatatgtactgggtgcgacaggctccaggcaagggactggagtgggtcgcatatatcagcaacgacggcgataatacttactatcctgacaccatccgggggagattcacaatctctagagataacagtaagaacactctgtacctgcagatgaactctctgagggcagaagacaccgccgtgtactattgcgcccgcgggaaatacgatggagcctggtttgcttattggggacagggcaccctggtgacagtcagctcc

SEQ ID NO: 12 - protein, 119 aa, Artificial sequence
  FG27 RHA
QVQLVESGGGVVQPGRSLRLSCAASGFTFSHYYMYWVRQAPGKGLEWVAYISNDGDNTYYPDTIRGRFTISRDNSKNTLYLQMNSLRAEDTAVYYCARGKYDGAWFAYWGQGTLVTVSS

SEQ ID NO: 13 - DNA, 990 bp, Artificial sequence
  HuG1 DNA sequence
gcctccaccaagggcccttccgtgttccctctggccccttcctccaagtccacctccggcggcaccgccgctctgggctgcctggtgaaggactacttccctgagcctgtgaccgtgtcctggaactctggcgccctgaccagcggcgtgcacaccttccctgccgtgctgcagtcctccggcctgtactccctgtcctccgtggtgaccgtgccttcctcctccctgggcacccagacctacatctgcaacgtgaaccacaagccttccaacaccaaggtggacaagaaggtggagcctaagtcctgcgacaagacccacacgtgccctccatgcccagctcccgagctgctgggcggaccaagcgtgtttctgttccctcctaagcctaaggacaccctgatgatctcccggacccctgaggtgacgtgcgtggtggtggacgtgtcccacgaggacccagaggtgaagttcaattggtacgtggacggcgtggaggtgcacaacgccaagaccaagcctcgggaggaacagtacaactccacctaccgggtggtgtctgtgctgaccgtgctgcaccaggactggctgaacggcaaggaatacaagtgcaaagtctccaacaaggccctgcctgcccccatcgaaaagaccatctccaaggccaagggccagcctcgcgagcctcaggtgtacaccctgcctccaagcagggaggaaatgaccaagaaccaggtgtccctgacctgtctggtgaagggcttctacccttccgatatcgccgtggagtgggagtccaacggccagcctgagaacaactacaagaccacccctcctgtgctggactccgacggctccttcttcctgtactccaagctgaccgtggacaagtcccggtggcagcagggcaacgtgttctcctgctccgtgatgcacgaggccctgcacaaccactacacccagaagagcctctccctgtccccgggtaaa

SEQ ID NO: 14 - protein, 330 aa, Artificial sequence
  HuG1 protein sequence
ASTKGPSVFPLAPSSKSTSGGTAALGCLVKDYFPEPVTVSWNSGALTSGVHTFPAVLQSSGLYSLSSVVTVPSSSLGTQTYICNVNHKPSNTKVDKKVEPKSCDKTHTCPPCPAPELLGGPSVFLFPPKPKDTLMISRTPEVTCVVVDVSHEDPEVKFNWYVDGVEVHNAKTKPREEQYNSTYRVVSVLTVLHQDWLNGKEYKCKVSNKALPAPIEKTISKAKGQPREPQVYTLPPSREEMTKNQVSLTCLVKGFYPSDIAVEWESNGQPENNYKTTPPVLDSDGSFFLYSKLTVDKSRWQQGNVFSCSVMHEALHNHYTQKSLSLSPGK

SEQ ID NO: 15 - DNA, 396 bp, Artificial sequence
  FG27 RKC DNA sequence
atggaagccccagcgcagcttctcttcctcctgctactctggctccctgataccaccggagacgtcgtgatgacccagagcccactgagcctgcctgtgacacccggcgagcccgcaagtatttcctgtagaagttcccagattatcgtgcacactaacgggaatacctacctggagtggtatctgcagaagcccggccagagtcctcagctgctgatctacaaagtgagtaaccggttctcaggagtcccagaccggttcagcggctccgggtctggaaccgatttcacactgaagattagcagggtggaggccgaagacgtgggagtctactattgctttcagggctcccatgtccccttcacatttggccaggggaccaagctggaaatcaaa

SEQ ID NO: 16 - protein, 132 aa, Artificial sequence
  FG27 RKC protein sequence
MEAPAQLLFLLLLWLPDTTGDVVMTQSPLSLPVTPGEPASISCRSSQIIVHTNGNTYLEWYLQKPGQSPQLLIYKVSNRFSGVPDRFSGSGSGTDFTLKISRVEAEDVGVYYCFQGSHVPFTFGQGTKLEIK

SEQ ID NO: 17 - DNA, 321 bp, Artificial sequence
  HuK DNA sequence
agaactgtggcagcaccaagcgtcttcatcttcccgccatctgatgagcagttgaaatctggaactgcctctgttgtgtgcctgctgaataacttctatcccagagaggccaaagtacagtggaaggtggataacgccctccaatcgggtaactcccaggagagtgtcacagagcaggacagcaaggacagcacctacagcctcagcagcaccctgacgctgagcaaagcagactacgagaaacacaaagtctacgcctgcgaagtcacccatcagggcctgagctcgcccgtcacaaagagcttcaacaggggagagtgt

SEQ ID NO: 18 - protein, 107 aa, Artificial sequence [sequence omitted]

SEQ ID NO: 19 - DNA, 714 bp, Artificial sequence; identical to SEQ ID NO: 9
  27 Light chain DNA sequence (variable region + Kappa constant)

SEQ ID NO: 20 - protein, 238 aa, Artificial sequence; identical to SEQ ID NO: 10
  27 Light chain protein sequence (variable region + Kappa constant)

SEQ ID NO: 21 - DNA, 1404 bp, Artificial sequence
  Heavy chain DNA sequence of i27v1 (variable + 'improved' v1 constant region)
atgaacttctggctcagcttgattttccttgtccttgttttaaaaggtgtccagtgtgaagtgaagctggtggagtctgggggaggcttagtgcagcctggagggtccctgaaactctcctgtgcaacctctggattcactttcagtcactattacatgtattgggttcgccagactccagagaagaggctggagtgggtcgcatacattagtaatgatggtgataacacctattatccagacactataaggggccgattcaccatctccagagacaatgccaggaacaccctgtacctgcaaatgagccgtctgaagtctgaggacacagccatgtattactgtgcaagagggaagtacgacggggcctggtttgcttactggggccaagggactctggtcactgtctctagcgcttccaccaagggcccatcggtcttccccctggcaccctcctccaagagcacctctgggggcacagcggccctgggctgcctggtcaaggactacttccccgaaccggtgacggtgtcgtggaactcaggcgccctgaccagcggcgtgcacaccttcccggctgtcctacagtcctcaggactctactccctcagcagcgtggtgaccgtgccctccagcagcttgggcacccagacctacatctgcaacgtgaatcacaagcccagcaacaccaaggtggacaagaaagttgagcccaaatcttgtgacaaaactcacacatgcccaccgtgcccagcacctgaactcctggggggaccgtcagtcttcctcttccccccaaaacccaaggacaccctcatgatctcccggacccctgaggtcacatgcgtggtggtggacgtgagccacgaagaccctgaggtcaagttcaactggtacgtggacggcgtggaggtgcatacagcctggacacagccccgtgaagagcagtacaacagtacctaccgagtggtcagtgtcctcaccgtcctgcaccaggactggctgaatggcaaggagtacaagtgcaaggtctccaacaaagccctcccagcccccatcgagaaaaccatctccaaacccaaaggaagagcccagacacctcaagtatacaccatacccccacctcgtgaacaaatgtccaagaagaaggttagtctgacctgcctggtcaccaacttcttctctgaagccatcagtgtggagtgggagagcaatgggcagccggagaacaactacaagaccacgcctcccgtgctggactccgacggctccttcttcctctacagcaagctcaccgtggacaagagcaggtggcagcaggggaacgtcttctcatgctccgtgatgcatgaggctctgcacaaccactacacgcagaagagcctctccctgtctccgggtaaa

SEQ ID NO: 22 - protein, 468 aa, Artificial sequence
  Heavy chain Protein sequence of i27v1 (variable + 'improved' v1 constant region)
MNFWLSLIFLVLVLKGVQCEVKLVESGGGLVQPGGSLKLSCATSGFTFSHYYMYWVRQTPEKRLEWVAYISNDGDNTYYPDTIRGRFTISRDNARNTLYLQMSRLKSEDTAMYYCARGKYDGAWFAYWGQGTLVTVSSASTKGPSVFPLAPSSKSTSGGTAALGCLVKDYFPEPVTVSWNSGALTSGVHTFPAVLQSSGLYSLSSVVTVPSSSLGTQTYICNVNHKPSNTKVDKKVEPKSCDKTHTCPPCPAPELLGGPSVFLFPPKPKDTLMISRTPEVTCVVVDVSHEDPEVKFNWYVDGVEVHTAWTQPREEQYNSTYRVVSVLTVLHQDWLNGKEYKCKVSNKALPAPIEKTISKPKGRAQTPQVYTIPPPREQMSKKKVSLTCLVTNFFSEAISVEWESNGQPENNYKTTPPVLDSDGSFFLYSKLTVDKSRWQQGNVFSCSVMHEALHNHYTQKSLSLSPGK